European Patent Application EP 4 748 384 A1, published May 27, 2026. Title: PREVENTION, TREATMENT AND/OR DIAGNOSIS OF ANAPHYLAXIS. Applicant: Fundación Instituto de Investigación Sanitaria Fundación Jiménez Díaz. The sequence listing filed with the application follows.

SEQUENCE LISTING (20 sequences)

SEQ ID NO: 1 - DNA, 19 bp, synthetic construct
  source 1..19: mol_type = other DNA
ctggagcgccaaatatgcg

SEQ ID NO: 2 - DNA, 21 bp, synthetic construct
  source 1..21: mol_type = other DNA
tgagactgtacggtagcaggt

SEQ ID NO: 3 - DNA, 21 bp, synthetic construct
  source 1..21: mol_type = other DNA
ccttgtcagggtagacagcct

SEQ ID NO: 4 - DNA, 22 bp, synthetic construct
  source 1..22: mol_type = other DNA
gacagaggtaaaagcagtctcg

SEQ ID NO: 5 - DNA, 24 bp, synthetic construct
  source 1..24: mol_type = other DNA
catctttgagagaactgaggtctt

SEQ ID NO: 6 - DNA, 21 bp, synthetic construct
  source 1..21: mol_type = other DNA
ccttcttcttcatgcggtaca

SEQ ID NO: 7 - DNA, 20 bp, synthetic construct
  source 1..20: mol_type = other DNA
cgccactttcatgaccgaga

SEQ ID NO: 8 - DNA, 24 bp, synthetic construct
  source 1..24: mol_type = other DNA
tcattcagaccgatccactggtag

SEQ ID NO: 9 - DNA, 19 bp, synthetic construct
  source 1..19: mol_type = other DNA
ggagagcgcactccatgac

SEQ ID NO: 10 - DNA, 21 bp, synthetic construct
  source 1..21: mol_type = other DNA
ctcagcatatacgtcccggaa

SEQ ID NO: 11 - DNA, 19 bp, synthetic construct
  source 1..19: mol_type = other DNA
tatgatgccgcccaagttg

SEQ ID NO: 12 - DNA, 23 bp, synthetic construct
  source 1..23: mol_type = other DNA
ctgttcaatttctcggacttcgt

SEQ ID NO: 13 - DNA, 21 bp, synthetic construct
  source 1..21: mol_type = other DNA
ctgctgattggtttcagtctt

SEQ ID NO: 14 - DNA, 21 bp, synthetic construct
  source 1..21: mol_type = other DNA
ccactgctactacagtctccc

SEQ ID NO: 15 - DNA, 21 bp, synthetic construct
  source 1..21: mol_type = other DNA
tcgatgctgacaccaattcaa

SEQ ID NO: 16 - DNA, 23 bp, synthetic construct
  source 1..23: mol_type = other DNA
tcccaatagacaagtgagaccaa

SEQ ID NO: 17 - DNA, 21 bp, synthetic construct
  source 1..21: mol_type = other DNA
gaaagggctgattgtgacccc

SEQ ID NO: 18 - DNA, 21 bp, synthetic construct
  source 1..21: mol_type = other DNA
agtagttccgcactgggtaca

SEQ ID NO: 19 - DNA, 21 bp, synthetic construct
  source 1..21: mol_type = other DNA
ccgtcgtagttccgaccataa

SEQ ID NO: 20 - DNA, 21 bp, synthetic construct
  source 1..21: mol_type = other DNA
cagctttgcaaccatactccc